European Patent Application EP 4 321 162 A1, published February 14, 2024. Title: ANTIVIRAL AGENTS FOR THE TREATMENT OF INFECTIONS BY CORONAVIRUSES. Applicant: CONSEJO SUPERIOR DE INVESTIGACIONES CIENTIFICAS CSIC. The sequence listing filed with the application follows.

SEQUENCE LISTING (23 sequences)

SEQ ID NO: 1 - protein, 4 aa, SARS CORONAVIRUS 2
DLLV

SEQ ID NO: 2 - protein, 4 aa, MERS CORONAVIRUS
DEWF

SEQ ID NO: 3 - DNA, 29 bp, synthetic construct
  source 1..29: mol_type = other DNA
ctcttcaggagttgctaatccagcaatgg

SEQ ID NO: 4 - DNA, 39 bp, synthetic construct
  source 1..39: mol_type = other DNA
ttagaaccattcatcaggaactccttcagaagagttcag

SEQ ID NO: 5 - DNA, 39 bp, synthetic construct; identical to SEQ ID NO: 4
  source 1..39: mol_type = other DNA

SEQ ID NO: 6 - DNA, 22 bp, synthetic construct
  source 1..22: mol_type = other DNA
ggtccttaatgtcacagcgccc

SEQ ID NO: 7 - DNA, 29 bp, synthetic construct
  source 1..29: mol_type = other DNA
ctcttcaggagttgctaatccagcaatgg

SEQ ID NO: 8 - DNA, 39 bp, synthetic construct
  source 1..39: mol_type = other DNA
cgtttagatcagatcatcaggaactccttcagaagagtt

SEQ ID NO: 9 - DNA, 42 bp, synthetic construct
  source 1..42: mol_type = other DNA
gaaggagttcctgatgatctgatctaaacgaactaactatta

SEQ ID NO: 10 - DNA, 22 bp, synthetic construct
  source 1..22: mol_type = other DNA
ggtccttaatgtcacagcgccc

SEQ ID NO: 11 - DNA, 29 bp, synthetic construct
  source 1..29: mol_type = other DNA
ctcttcaggagttgctaatccagcaatgg

SEQ ID NO: 12 - DNA, 34 bp, synthetic construct
  source 1..34: mol_type = other DNA
ttagacgtcatcaacaggaactccttcagaagag

SEQ ID NO: 13 - DNA, 45 bp, synthetic construct
  source 1..45: mol_type = other DNA
tctgaaggagttcctgttgatgacgtctaaacgaactaactatta

SEQ ID NO: 14 - DNA, 22 bp, synthetic construct
  source 1..22: mol_type = other DNA
ggtccttaatgtcacagcgccc

SEQ ID NO: 15 - DNA, 20 bp, synthetic construct
  source 1..20: mol_type = other DNA
gcttatcgtttaagcagctc

SEQ ID NO: 16 - DNA, 48 bp, synthetic construct
  source 1..48: mol_type = other DNA
catattagacattatgaaggagttcgttatcctcctcctccaggtggt

SEQ ID NO: 17 - DNA, 48 bp, synthetic construct
  source 1..48: mol_type = other DNA
aaccccctctaccacctggaggaggaggataacgaactccttcataat

SEQ ID NO: 18 - DNA, 20 bp, synthetic construct
  source 1..20: mol_type = other DNA
tctgtcgtagtcacaagcac

SEQ ID NO: 19 - protein, 76 aa, SARS CORONAVIRUS 2
MYSFVSEETGTLIVNSVLLFLAFVVFLLVTLAILTALRLCAYCCNIVNVSLVKPTVYVYSRVKNLNSSEGVPDLLV

SEQ ID NO: 20 - protein, 76 aa, synthetic construct
MYSFVSEETGTLIVNSVLLFLAFVVFLLVTLAILTALRLCAYCCNIVNVSLVKPTVYVYSRVKNLNSSEGVPDEWF

SEQ ID NO: 21 - protein, 76 aa, synthetic construct
MYSFVSEETGTLIVNSVLLFLAFVVFLLVTLAILTALRLCAYCCNIVNVSLVKPTVYVYSRVKNLNSSEGVPVDDV

SEQ ID NO: 22 - protein, 76 aa, synthetic construct
MYSFVSEETGTLIVNSVLLFLAFVVFLLVTLAILTALRLCAYCCNIVNVSLVKPTVYVYSRVKNLNSSEGVPDDLI

SEQ ID NO: 23 - protein, 76 aa, synthetic construct
MYSFVSEETGTLIVNSVLLFLAFVVFLLVTLAILTALRLCAYCCNIVNVSLVKPTVYVYSRVKNLNSSEGVPGGGG